European Patent Application EP 4 599 836 A1, published August 13, 2025. Title: Method for preventing and/or treating infections. Applicant: FUNDACIO INSTITUT DE BIOENGINYERIA DE CATALUNYA. Application EP. The sequence listing filed with the application follows.

SEQUENCE LISTING (26 sequences)

SEQ ID NO: 1 - DNA, 26 bp, Galleria mellonella
  source 1..26: mol_type = other DNA
aaggatccgcggttcgcgacgccgtc

SEQ ID NO: 2 - DNA, 28 bp, Galleria mellonella
  source 1..28: mol_type = other DNA
aagggcccagcgccttgtaggtcgcgtt

SEQ ID NO: 3 - DNA, 20 bp, Galleria mellonella
  source 1..20: mol_type = other DNA
atggttgcaaagctgaaact

SEQ ID NO: 4 - DNA, 20 bp, Galleria mellonella
  source 1..20: mol_type = other DNA
tcccgtgttgagtcaaatta

SEQ ID NO: 5 - DNA, 20 bp, Galleria mellonella
  source 1..20: mol_type = other DNA
agacttgcacgccatcaaga

SEQ ID NO: 6 - DNA, 20 bp, Galleria mellonella
  source 1..20: mol_type = other DNA
tgcatgctgtttgtcactgc

SEQ ID NO: 7 - DNA, 18 bp, Galleria mellonella
  source 1..18: mol_type = other DNA
agatgcacggtcctacag

SEQ ID NO: 8 - DNA, 18 bp, Galleria mellonella
  source 1..18: mol_type = other DNA
gatcgtaggtgccttgtg

SEQ ID NO: 9 - DNA, 20 bp, Galleria mellonella
  source 1..20: mol_type = other DNA
tcccaactcttgaccgacga

SEQ ID NO: 10 - DNA, 20 bp, Galleria mellonella
  source 1..20: mol_type = other DNA
agtggttgcgccatccatac

SEQ ID NO: 11 - DNA, 17 bp, Galleria mellonella
  source 1..17: mol_type = other DNA
ctgcgccatgttcttca

SEQ ID NO: 12 - DNA, 19 bp, Galleria mellonella
  source 1..19: mol_type = other DNA
tcgcatctctgatcctctg

SEQ ID NO: 13 - DNA, 20 bp, Galleria mellonella
  source 1..20: mol_type = other DNA
gctgtactcgctgcactgat

SEQ ID NO: 14 - DNA, 20 bp, Galleria mellonella
  source 1..20: mol_type = other DNA
tggcgatcattgccctcttt

SEQ ID NO: 15 - DNA, 20 bp, Galleria mellonella
  source 1..20: mol_type = other DNA
cccgaagacgctggtgaata

SEQ ID NO: 16 - DNA, 20 bp, Galleria mellonella
  source 1..20: mol_type = other DNA
cgcacgttcatttgctgttc

SEQ ID NO: 17 - DNA, 20 bp, Galleria mellonella
  source 1..20: mol_type = other DNA
gacagaagtcctccggtcag

SEQ ID NO: 18 - DNA, 20 bp, Galleria mellonella
  source 1..20: mol_type = other DNA
tccgtcttcaagcaaaggca

SEQ ID NO: 19 - DNA, 20 bp, Galleria mellonella
  source 1..20: mol_type = other DNA
tggcacggcatcagttatca

SEQ ID NO: 20 - DNA, 20 bp, Galleria mellonella
  source 1..20: mol_type = other DNA
acagcgactgtcatgtggaa

SEQ ID NO: 21 - DNA, 21 bp, Galleria mellonella
  source 1..21: mol_type = other DNA
atgaaggtgctgaagtcacaa

SEQ ID NO: 22 - DNA, 21 bp, Galleria mellonella
  source 1..21: mol_type = other DNA
gccattttacaatcgccacaa

SEQ ID NO: 23 - DNA, 20 bp, Galleria mellonella
  source 1..20: mol_type = other DNA
atttgtaacggtggacacga

SEQ ID NO: 24 - DNA, 19 bp, Galleria mellonella
  source 1..19: mol_type = other DNA
cgcaaattggtatgcatgg

SEQ ID NO: 25 - DNA, 19 bp, Galleria mellonella
  source 1..19: mol_type = other DNA
cccgaagatgaacgatcac

SEQ ID NO: 26 - DNA, 20 bp, Galleria mellonella
  source 1..20: mol_type = other DNA
cgaaaggcctagaacgtttg